European Patent Application EP 4 450 620 A1, published October 23, 2024. Title: 可控合成单链DNA的末端转移酶变体及应用. Applicant: 中国科学院天津工业生物技术研究所. The sequence listing filed with the application follows.

SEQUENCE LISTING (4 sequences)

SEQ ID NO: 1 - protein, 513 aa, Zonotrichia albicollis
MDRFKAPAVISQRKRQKGLHSPKLSCSYEIKFSNFVIFIMQRKMGLTRRMFLMELGRRKGFRVESELSDSVTHIVAENNSYLEVLDWLKGQAVGDSSRFELLDISWFTACMEAGRPVDSEVKYRLMEQSQSLPLNMPALEMPAFIATKVSQYSCQRKTTLNNYNKKFTDAFEVMAENYEFKENEIFCLEFLRAASLLKSLPFSVTRMKDIQGLPCVGDQVRDIIEEIIEEGESSRVNEVLNDERYKAFKQFTSVFGVGVKTSEKWYRMGLRTVEEVKADKTLKLSKMQKAGLLYYEDLVSCVSKAEADAVSLIVKNTVCTFLPDALVTITGGFRRGKNIGHDIDFLITNPGPREDDELLHKVIDLWKKQGLLLYCDIIESTFVKEQLPSRKVDAMDHFQKCFAILKLYQPRVDNSTCNTSEQLEMAEVKDWKAIRVDLVITPFEQYPYALLGWTGSRQFGRDLRRYAAHERKMILDNHGLYDRRKRIFLKAGSEEEIFAHLGLDYVEPWERNA

SEQ ID NO: 2 - protein, 382 aa, Zonotrichia albicollis
LPLNMPALEMPAFIATKVSQYSCQRKTTLNNYNKKFTDAFEVMAENYEFKENEIFCLEFLRAASLLKSLPFSVTRMKDIQGLPCVGDQVRDIIEEIIEEGESSRVNEVLNDERYKAFKQFTSVFGVGVKTSEKWYRMGLRTVEEVKADKTLKLSKMQKAGLLYYEDLVSCVSKAEADAVSLIVKNTVCTFLPDALVTITGGFRRGKNIGHDIDFLITNPGPREDDELLHKVIDLWKKQGLLLYCDIIESTFVKEQLPSRKVDAMDHFQKCFAILKLYQPRVDNSTCNTSEQLEMAEVKDWKAIRVDLVITPFEQYPYALLGWTGSRQFGRDLRRYAAHERKMILDNHGLYDRRKRIFLKAGSEEEIFAHLGLDYVEPWERNA

SEQ ID NO: 3 - protein, 896 aa, Zonotrichia albicollis
MKIEEGKLVIWINGDKGYNGLAEVGKKFEKDTGIKVTVEHPDKLEEKFPQVAATGDGPDIIFWAHDRFGGYAQSGLLAEITPDKAFQDKLYPFTWDAVRYNGKLIAYPIAVEALSLIYNKDLLPNPPKTWEEIPALDKELKAKGKSALMFNLQEPYFTWPLIAADGGYAFKYENGKYDIKDVGVDNAGAKAGLTFLVDLIKNKHMNADTDYSIAEAAFNKGETAMTINGPWAWSNIDTSKVNYGVTVLPTFKGQPSKPFVGVLSAGINAASPNKELAKEFLENYLLTDEGLEAVNKDKPLGAVALKSYEEELVKDPRIAATMENAQKGEIMPNIPQMSAFWYAVRTAVINAASGRQTVDEALKDAQTNSSSNNNNNNNNNNLGMDRFKAPAVISQRKRQKGLHSPKLSCSYEIKFSNFVIFIMQRKMGLTRRMFLMELGRRKGFRVESELSDSVTHIVAENNSYLEVLDWLKGQAVGDSSRFELLDISWFTACMEAGRPVDSEVKYRLMEQSQSLPLNMPALEMPAFIATKVSQYSCQRKTTLNNYNKKFTDAFEVMAENYEFKENEIFCLEFLRAASLLKSLPFSVTRMKDIQGLPCVGDQVRDIIEEIIEEGESSRVNEVLNDERYKAFKQFTSVFGVGVKTSEKWYRMGLRTVEEVKADKTLKLSKMQKAGLLYYEDLVSCVSKAEADAVSLIVKNTVCTFLPDALVTITGGFRRGKNIGHDIDFLITNPGPREDDELLHKVIDLWKKQGLLLYCDIIESTFVKEQLPSRKVDAMDHFQKCFAILKLYQPRVDNSTCNTSEQLEMAEVKDWKAIRVDLVITPFEQYPYALLGWTGSRQFGRDLRRYAAHERKMILDNHGLYDRRKRIFLKAGSEEEIFAHLGLDYVEPWERNA

SEQ ID NO: 4 - protein, 765 aa, Zonotrichia albicollis
MKIEEGKLVIWINGDKGYNGLAEVGKKFEKDTGIKVTVEHPDKLEEKFPQVAATGDGPDIIFWAHDRFGGYAQSGLLAEITPDKAFQDKLYPFTWDAVRYNGKLIAYPIAVEALSLIYNKDLLPNPPKTWEEIPALDKELKAKGKSALMFNLQEPYFTWPLIAADGGYAFKYENGKYDIKDVGVDNAGAKAGLTFLVDLIKNKHMNADTDYSIAEAAFNKGETAMTINGPWAWSNIDTSKVNYGVTVLPTFKGQPSKPFVGVLSAGINAASPNKELAKEFLENYLLTDEGLEAVNKDKPLGAVALKSYEEELVKDPRIAATMENAQKGEIMPNIPQMSAFWYAVRTAVINAASGRQTVDEALKDAQTNSSSNNNNNNNNNNLGLPLNMPALEMPAFIATKVSQYSCQRKTTLNNYNKKFTDAFEVMAENYEFKENEIFCLEFLRAASLLKSLPFSVTRMKDIQGLPCVGDQVRDIIEEIIEEGESSRVNEVLNDERYKAFKQFTSVFGVGVKTSEKWYRMGLRTVEEVKADKTLKLSKMQKAGLLYYEDLVSCVSKAEADAVSLIVKNTVCTFLPDALVTITGGFRRGKNIGHDIDFLITNPGPREDDELLHKVIDLWKKQGLLLYCDIIESTFVKEQLPSRKVDAMDHFQKCFAILKLYQPRVDNSTCNTSEQLEMAEVKDWKAIRVDLVITPFEQYPYALLGWTGSRQFGRDLRRYAAHERKMILDNHGLYDRRKRIFLKAGSEEEIFAHLGLDYVEPWERNA